European Patent Specification EP 4 359 557 B1, published May 20, 2026. Title: METHODS AND COMPOSITIONS FOR COMBINATORIAL INDEXING OF BEAD-BASED NUCLEIC ACIDS. Applicant: Manzo, Andrea Brown, Colin Norberg, Steven Harrington, Timothy. The sequence listing filed with the application follows.

SEQUENCE LISTING (14 sequences)

SEQ ID NO: 1 - DNA, 20 bp, Artificial Sequence
  Artificial oligonucleotides
aatgatacggcgaccaccga

SEQ ID NO: 2 - DNA, 24 bp, Artificial Sequence
  Artificial oligonucleotides
caagcagaagacggcatacgagat

SEQ ID NO: 3 - DNA, 16 bp, Artificial Sequence
  Artificial oligonucleotides
atgctctagacaagtc

SEQ ID NO: 4 - DNA, 12 bp, Artificial Sequence
  Artificial oligonucleotides
tgctctacaagc

SEQ ID NO: 5 - DNA, 12 bp, Artificial Sequence
  Artificial oligonucleotides
gctctaacaagc

SEQ ID NO: 6 - DNA, 12 bp, Artificial Sequence
  Artificial oligonucleotides
gctctaacaagc

SEQ ID NO: 7 - DNA, 14 bp, Artificial Sequence
  Artificial oligonucleotides
gacttgtccggtgg

SEQ ID NO: 8 - DNA, 14 bp, Artificial Sequence
  Artificial oligonucleotides
ctgaacaggccacc

SEQ ID NO: 9 - DNA, 12 bp, Artificial Sequence
  Artificial oligonucleotides
ctgaacaggcca

SEQ ID NO: 10 - DNA, 12 bp, Artificial Sequence
  Artificial oligonucleotides
gaacaggccacc

SEQ ID NO: 11 - DNA, 15 bp, Artificial Sequence
  Artificial oligonucleotides
  misc_feature 15: N is inosine
ctgaacaggccaccn

SEQ ID NO: 12 - DNA, 16 bp, Artificial Sequence
  CTGAACAGGCCACCNN
  misc_feature 15, 16: N is Inosine
ctgaacaggccaccnn

SEQ ID NO: 13 - DNA, 14 bp, Artificial Sequence
  Artificial oligonucleotides
  misc_feature 13, 14: N is inosine
ctgaacaggccann

SEQ ID NO: 14 - DNA, 16 bp, Artificial Sequence
  Artificial oligonucleotides
  misc_feature 13, 14, 15, 16: N is inosine
ctgaacaggccannnn